European Patent Specification EP 3 402 457 B1, published February 25, 2026. Title: PROTEIN CAGE-STABILIZED PICKERING EMULSIONS AND THE USE THEREOF. Applicant: NANYANG TECHNOLOGICAL UNIVERSITY AGENCY FOR SCIENCE, TECHNOLOGY AND RESEARCH. Application 17738735.4. The sequence listing filed with the application follows.

SEQUENCE LISTING (6 sequences)

SEQ ID NO: 1 - protein, 260 aa, Bacillus stearothermophilus
MLSVPGPAAAEEKAAPAAAKPATTEGEFPETREKMSGIRRAIAKAMVHSKHTAPHVTLMDEADVTKLVAHRKKFKAIAAEKGIKLTFLPYVVKALVSALREYPVLNTSIDDETEEIIQKHYYNIGIAADTDRGLLVPVIKHADRKPIFALAQEINELAEKARDGKLTPGEMKGASCTITNIGSAGGQWFTPVINHPEVAILGIGRIAEKPIVRDGEIVAAPMLALSLSFDHRMIDGATAQKALNHIKRLLSDPELLLMEA

SEQ ID NO: 2 - protein, 260 aa, Bacillus stearothermophilus
MLSVPGPAAAEEKAAPAAAKPATTEGEFPETREKMSGIRRAIAKAMVHSKHTAPHVTLMDEADVTKLVAHRKKFKAIAAEKGIKLTFLPYVVKALVSALREYPVLNTSIDDETEEIIQKHYYNIGIAADTDRGLLVPVIKHADRKPIFALAQEINELAEKARDGKLTPGEMKGASCTITNIGSAGGQWFTPVINHPEVAILGIGRIAEKPIVRCCEIVAAPMLALSLSFDHRMIDGATAQKALNHIKRLLSDPELLLMEA

SEQ ID NO: 3 - protein, 173 aa, Archaeoglobus fulgidus
MASISEKMVEALNRQINAEIYSAYLYLSMASYFDSIGLKGFSNWMRVQWQEELMHAMKMFDFVSERGGRVKLYAVEEPPSEWDSPLAAFEHVYEHEVNVTKRIHELVEMAMQEKDFATYNFLQWYVAEQVEEEASALDIVEKLRLIGEDKRALLFLDKELSLRQFTPPAEEEK

SEQ ID NO: 4 - protein, 170 aa, Archaeoglobus fulgidus
MASISEKMVEALNRQINAEIYSAYLYLSMASYFDSIGLKGFSNWMRVQWQEELMHAMKMFDFVSERGGRVKLYAVEEPPSEWDSPLAAFEHVYEHEVNVTKRIHELVEMAMQEKDFATYNFLQWYVAEQVEEEASALDIVEKLRLIGEDAAALLFLDKELSLRQFTPPAE

SEQ ID NO: 5 - protein, 183 aa, Homo sapiens
MTTASTSQVRQNYHQDSEAAINRQINLELYASYVYLSMSYYFDRDDVALKNFAKYFLHQSHEEREHAEKLMKLQNQRGGRIFLQDIKKPDCDDWESGLNAMECALHLEKNVNQSLLELHKLATDKNDPHLCDFIETHYLNEQVKAIKELGDHVTNLRKMGAPESGLAEYLFDKHTLGDSDNES

SEQ ID NO: 6 - protein, 175 aa, Homo sapiens
MSSQIRQNYSTDVEAAVNSLVNLYLQASYTYLSLGFYFDRDDVALEGVSHFFRELAEEKREGYERLLKMQNQRGGRALFQDIKKPAEDEWGKTPDAMKAAMALEKKLNQALLDLHALGSARTDPHLCDFLETHFLDEEVKLIKKMGDHLTNLHRLGGPEAGLGEYLFERLTLKHD